European Patent Specification EP 3 851 459 B1, published May 1, 2024. Title: MULTIMERIC IL-15 SOLUBLE FUSION MOLECULES AND METHODS OF MAKING AND USING SAME. Applicant: ALTOR BIOSCIENCE CORPORATION. The sequence listing filed with the application follows.

SEQUENCE LISTING (51 sequences)

SEQ ID NO: 1 - protein, 6 aa, Homo sapiens
PELLGG

SEQ ID NO: 2 - protein, 6 aa, Homo sapiens
PEAAGG

SEQ ID NO: 3 - protein, 5 aa, Homo sapiens
KCKSL

SEQ ID NO: 4 - protein, 5 aa, Homo sapiens
KCASL

SEQ ID NO: 5 - protein, 10 aa, Artificial Sequence
  source: /note="Description of Artificial Sequence: Synthetic peptide"
ASGGGGSGGG

SEQ ID NO: 6 - DNA, 25 bp, Artificial Sequence
  source: /note="Description of Artificial Sequence: Synthetic primer"
tgttgggaattcatcacgtgccctc

SEQ ID NO: 7 - DNA, 32 bp, Artificial Sequence
  source: /note="Description of Artificial Sequence: Synthetic primer"
tggtgtgaattctctaatgcatttgagactgg

SEQ ID NO: 8 - DNA, 53 bp, Artificial Sequence
  source: /note="Description of Artificial Sequence: Synthetic primer"
gtacgacttaattaactcgagccaccatggagacagacacactcctgttatgg

SEQ ID NO: 9 - DNA, 33 bp, Artificial Sequence
  source: /note="Description of Artificial Sequence: Synthetic primer"
cttcccgttaacccaccagctcagctccacgtg

SEQ ID NO: 10 - DNA, 37 bp, Artificial Sequence
  source: /note="Description of Artificial Sequence: Synthetic primer"
ctggtgggttaacgggaaggaggtgcacagtggggtc

SEQ ID NO: 11 - DNA, 34 bp, Artificial Sequence
  source: /note="Description of Artificial Sequence: Synthetic primer"
gagggcacgtgatgtctgctctaccccaggcctc

SEQ ID NO: 12 - DNA, 32 bp, Artificial Sequence
  source: /note="Description of Artificial Sequence: Synthetic primer"
gtagagcagacatcacgtgccctccccccatg

SEQ ID NO: 13 - DNA, 42 bp, Artificial Sequence
  source: /note="Description of Artificial Sequence: Synthetic primer"
ccttggtgctagctctaatacatttgagactgggggttgtcc

SEQ ID NO: 14 - DNA, 44 bp, Artificial Sequence
  source: /note="Description of Artificial Sequence: Synthetic primer"
ccagtctcaaatgtattagagctagcaccaagggcccatcggtc

SEQ ID NO: 15 - DNA, 52 bp, Artificial Sequence
  source: /note="Description of Artificial Sequence: Synthetic primer"
gtaatattctagacgcgttcattatttaccaggagacagggagaggctcttc

SEQ ID NO: 16 - DNA, 44 bp, Artificial Sequence
  source: /note="Description of Artificial Sequence: Synthetic primer"
gacttcaagcttaattaagccaccatggacagacttacttcttc

SEQ ID NO: 17 - DNA, 30 bp, Artificial Sequence
  source: /note="Description of Artificial Sequence: Synthetic primer"
cacccagttgtctgctctaccccaggcctc

SEQ ID NO: 18 - DNA, 43 bp, Artificial Sequence
  source: /note="Description of Artificial Sequence: Synthetic primer"
ctggggtagagcagacaactgggtgaatgtaataagtgatttg

SEQ ID NO: 19 - DNA, 49 bp, Artificial Sequence
  source: /note="Description of Artificial Sequence: Synthetic primer"
cctcatgcattcgaatccggatcattaagaagtgttgatgaacatttgg

SEQ ID NO: 20 - protein, 8 aa, Gallus gallus
SIINFEKL

SEQ ID NO: 21 - protein, 20 aa, Artificial Sequence
  source: /note="Description of Artificial Sequence: Synthetic peptide"
GGGGSGGGGSGGGGSGGGGS

SEQ ID NO: 22 - DNA, 53 bp, Artificial Sequence
  source: /note="Description of Artificial Sequence: Synthetic primer"
gtgagttttgtcacaagatttcggctctctaatgcatttgagactgggggttg

SEQ ID NO: 23 - DNA, 27 bp, Artificial Sequence
  source: /note="Description of Artificial Sequence: Synthetic primer"
gagccgaaatcttgtgacaaaactcac

SEQ ID NO: 24 - protein, 9 aa, Homo sapiens
STPPPGTRV

SEQ ID NO: 25 - protein, 9 aa, Homo sapiens
LLGRNSFEV

SEQ ID NO: 26 - protein, 8 aa, Vesicular stomatitis virus
RGYVYQGL

SEQ ID NO: 27 - protein, 25 aa, Artificial Sequence
  source: /note="Description of Artificial Sequence: Synthetic peptide"
DTSGGGGSGGGGSGGGGSGGGGSSS

SEQ ID NO: 28 - protein, 25 aa, Artificial Sequence
  source: /note="Description of Artificial Sequence: Synthetic peptide"
TSGGGGSGGGGSPGGGGSGGGGSSS

SEQ ID NO: 29 - protein, 25 aa, Artificial Sequence
  source: /note="Description of Artificial Sequence: Synthetic peptide"
DTSGGGGSGGGASGGGGSGGGGSSS

SEQ ID NO: 30 - protein, 21 aa, Artificial Sequence
  source: /note="Description of Artificial Sequence: Synthetic peptide"
SGGGGSGGGASGGGGSGGGGS

SEQ ID NO: 31 - protein, 19 aa, Artificial Sequence
  source: /note="Description of Artificial Sequence: Synthetic peptide"
VNEPKSSDKTHTSPPSPTR

SEQ ID NO: 32 - protein, 12 aa, Artificial Sequence
  source: /note="Description of Artificial Sequence: Synthetic peptide"
SGGGSGGGGSID

SEQ ID NO: 33 - protein, 21 aa, Artificial Sequence
  source: /note="Description of Artificial Sequence: Synthetic peptide"
SGGGGSGGGGSGGGGSGGGGS

SEQ ID NO: 34 - DNA, 2397 bp, Artificial Sequence
  source: /note="Description of Artificial Sequence: Synthetic polynucleotide"
atggacagacttacttcttcattcctgctcctgattgtccctgcgtacgtcttgtcccagtcagtgacgcagcccgatgctcgcgtcactgtctctgaaggagcctctctgcagctgagatgcaagtattcctactctgggacaccttatctgttctggtatgtccagtacccgcggcaggggctgcagctgctcctcaagtactattcaggagacccagtggttcaaggagtgaatggcttcgaggctgagttcagcaagagtaactcttccttccacctgcggaaagcctctgtgcactggagcgactctgctgtgtacttctgtgttttgagcgaggatagcaactatcagttgatctggggctctgggaccaagctaattataaagccagacactagtggtggcggtggcagcggcggtggtggttccggtggcggcggttctggcggtggcggttcctcgagcaattcaaaagtcattcagactccaagatatctggtgaaagggcaaggacaaaaagcaaagatgaggtgtatccctgaaaagggacatccagttgtattctggtatcaacaaaataagaacaatgagtttaaatttttgattaactttcagaatcaagaagttcttcagcaaatagacatgactgaaaaacgattctctgctgagtgtccttcaaactcaccttgcagcctagaaattcagtcctctgaggcaggagactcagcactgtacctctgtgccagcagtctgtcagggggcggcacagaagttttctttggtaaaggaaccaggctcacagttgtagaggacctgaacaaggtgttcccacccgaggtcgctgtgtttgagccatcagaagcagagatctcccacacccaaaaggccacactggtgtgcctggccacaggcttcttccctgaccacgtggagctgagctggtgggtgaatgggaaggaggtgcacagtggggtcagcacggacccgcagcccctcaaggagcagcccgccctcaatgactccagatactgcctgagcagccgcctgagggtctcggccaccttctggcagaacccccgcaaccacttccgctgtcaagtccagttctacgggctctcggagaatgacgagtggacccaggatagggccaaacccgtcacccagatcgtcagcgccgaggcctggggtagagcagacgaattcatcacgtgccctccccccatgtccgtggaacacgcagacatctgggtcaagagctacagcttgtactccagggagcggtacatttgtaactctggtttcaagcgtaaagccggcacgtccagcctgacggagtgcgtgttgaacaaggccacgaatgtcgcccactggacaacccccagtctcaaatgcattagagaattcgcctccaccaagggcccatcggtcttccccctggcaccctcctccaagagcacctctgggggcacagcggccctgggctgcctggtcaaggactacttccccgaaccggtgacggtgtcgtggaactcaggcgccctgaccagcggcgtgcacaccttcccggctgtcctacagtcctcaggactctactccctcagcagcgtggtgaccgtgccctccagcagcttgggcacccagacctacatctgcaacgtgaatcacaagcccagcaacaccaaggtggacaagaaagttgagcccaaatcttgtgacaaaactcacacatgcccaccgtgcccagcacctgaactcctggggggaccgtcagtcttcctcttccccccaaaacccaaggacaccctcatgatctcccggacccctgaggtcacatgcgtggtggtggacgtgagccacgaagaccctgaggtcaagttcaactggtacgtggacggcgtggaggtgcataatgccaagacaaagccgcgggaggagcagtacaacagcacgtaccgtgtggtcagcgtcctcaccgtcctgcaccaggactggctgaatggcaaggagtacaagtgcaaggtctccaacaaagccctcccagcccccatcgagaaaaccatctccaaagccaaagggcagccccgagaaccacaggtgtacaccctgcccccatcccgggatgagctgaccaagaaccaggtcagcctgacctgcctggtcaaaggcttctatcccagcgacatcgccgtggagtgggagagcaatgggcagccggagaacaactacaagaccacgcctcccgtgctggactccgacggctccttcttcctctacagcaagctcaccgtggacaagagcaggtggcagcaggggaacgtcttctcatgctccgtgatgcatgaggctctgcacaaccactacacgcagaagagcctctccctgtctccgggtaaa

SEQ ID NO: 35 - protein, 799 aa, Artificial Sequence [sequence omitted]

SEQ ID NO: 36 - DNA, 2391 bp, Artificial Sequence
  source: /note="Description of Artificial Sequence: Synthetic polynucleotide"
atggagacagacacactcctgttatgggtactgctgctctgggttccaggttccaccggtcagtcagtgacgcagcccgatgctcgcgtcactgtctctgaaggagcctctctgcagctgagatgcaagtattcctactctgggacaccttatctgttctggtatgtccagtacccgcggcaggggctgcagctgctcctcaagtactattcaggagacccagtggttcaaggagtgaatggcttcgaggctgagttcagcaagagtaactcttccttccacctgcggaaagcctctgtgcactggagcgactctgctgtgtacttctgtgttttgagcgaggatagcaactatcagttgatctggggctctgggaccaagctaattataaagccagacactagtggtggcggtggcagcggcggtggtggttccggtggcggcggttctggcggtggcggttcctcgagcaattcaaaagtcattcagactccaagatatctggtgaaagggcaaggacaaaaagcaaagatgaggtgtatccctgaaaagggacatccagttgtattctggtatcaacaaaataagaacaatgagtttaaatttttgattaactttcagaatcaagaagttcttcagcaaatagacatgactgaaaaacgattctctgctgagtgtccttcaaactcaccttgcagcctagaaattcagtcctctgaggcaggagactcagcactgtacctctgtgccagcagtctgtcagggggcggcacagaagttttctttggtaaaggaaccaggctcacagttgtagaggacctgaacaaggtgttcccacccgaggtcgctgtgtttgagccatcagaagcagagatctcccacacccaaaaggccacactggtgtgcctggccacaggcttcttccctgaccacgtggagctgagctggtgggttaacgggaaggaggtgcacagtggggtcagcacggacccgcagcccctcaaggagcagcccgccctcaatgactccagatactgcctgagcagccgcctgagggtctcggccaccttctggcagaacccccgcaaccacttccgctgtcaagtccagttctacgggctctcggagaatgacgagtggacccaggatagggccaaacccgtcacccagatcgtcagcgccgaggcctggggtagagcagacatcacgtgccctccccccatgtccgtggaacacgcagacatctgggtcaagagctacagcttgtactccagggagcggtacatttgtaactctggtttcaagcgtaaagccggcacgtccagcctgacggagtgcgtgttgaacaaggccacgaatgtcgcccactggacaacccccagtctcaaatgtattagagctagcaccaagggcccatcggtcttccccctggcaccctcctccaagagcacctctgggggcacagcggccctgggctgcctggtcaaggactacttccccgaaccggtgacggtgtcgtggaactcaggcgccctgaccagcggcgtgcacaccttcccggctgtcctacagtcctcaggactctactccctcagcagcgtggtgaccgtgccctccagcagcttgggcacccagacctacatctgcaacgtgaatcacaagcccagcaacaccaaggtggacaagaaagttgagcccaaatcttgtgacaaaactcacacatgcccaccgtgcccagcacctgaactcctggggggaccgtcagtcttcctcttccccccaaaacccaaggacaccctcatgatctcccggacccctgaggtcacatgcgtggtggtggacgtgagccacgaagaccctgaggtcaagttcaactggtacgtggacggcgtggaggtgcataatgccaagacaaagccgcgggaggagcagtacaacagcacgtaccgtgtggtcagcgtcctcaccgtcctgcaccaggactggctgaatggcaaggagtacaagtgcaaggtctccaacaaagccctcccagcccccatcgagaaaaccatctccaaagccaaagggcagccccgagaaccacaggtgtacaccctgcccccatcccgggatgagctgaccaagaaccaggtcagcctgacctgcctggtcaaaggcttctatcccagcgacatcgccgtggagtgggagagcaatgggcagccggagaacaactacaagaccacgcctcccgtgctggactccgacggctccttcttcctctacagcaagctcaccgtggacaagagcaggtggcagcaggggaacgtcttctcatgctccgtgatgcatgaggctctgcacaaccactacacgcagaagagcctctccctgtctccgggtaaataa

SEQ ID NO: 37 - protein, 796 aa, Artificial Sequence
  source: /note="Description of Artificial Sequence: Synthetic polypeptide"
METDTLLLWVLLLWVPGSTGQSVTQPDARVTVSEGASLQLRCKYSYSGTPYLFWYVQYPRQGLQLLLKYYSGDPVVQGVNGFEAEFSKSNSSFHLRKASVHWSDSAVYFCVLSEDSNYQLIWGSGTKLIIKPDTSGGGGSGGGGSGGGGSGGGGSSSNSKVIQTPRYLVKGQGQKAKMRCIPEKGHPVVFWYQQNKNNEFKFLINFQNQEVLQQIDMTEKRFSAECPSNSPCSLEIQSSEAGDSALYLCASSLSGGGTEVFFGKGTRLTVVEDLNKVFPPEVAVFEPSEAEISHTQKATLVCLATGFFPDHVELSWWVNGKEVHSGVSTDPQPLKEQPALNDSRYCLSSRLRVSATFWQNPRNHFRCQVQFYGLSENDEWTQDRAKPVTQIVSAEAWGRADITCPPPMSVEHADIWVKSYSLYSRERYICNSGFKRKAGTSSLTECVLNKATNVAHWTTPSLKCIRASTKGPSVFPLAPSSKSTSGGTAALGCLVKDYFPEPVTVSWNSGALTSGVHTFPAVLQSSGLYSLSSVVTVPSSSLGTQTYICNVNHKPSNTKVDKKVEPKSCDKTHTCPPCPAPELLGGPSVFLFPPKPKDTLMISRTPEVTCVVVDVSHEDPEVKFNWYVDGVEVHNAKTKPREEQYNSTYRVVSVLTVLHQDWLNGKEYKCKVSNKALPAPIEKTISKAKGQPREPQVYTLPPSRDELTKNQVSLTCLVKGFYPSDIAVEWESNGQPENNYKTTPPVLDSDGSFFLYSKLTVDKSRWQQGNVFSCSVMHEALHNHYTQKSLSLSPGK

SEQ ID NO: 38 - DNA, 1539 bp, Artificial Sequence
  source: /note="Description of Artificial Sequence: Synthetic polynucleotide"
atggacagacttacttcttcattcctgctcctgattgtccctgcgtacgtcttggcccagaaggtaacacagactcagacttcaatttctgtgatggagaagacaacggtgacaatggactgtgtgtatgaaacccgggacagttcttacttcttattctggtacaagcaaacagcaagtggggaaatagttttccttattcgtcaggactcttacaaaaaggaaaatgcaacagaaggtcattattctctgaactttcagaagccaaaaagttccatcggactcatcatcactgccacacagattgaggactcagcagtatatttctgtgctatgagagacacaaatgcttacaaagtcatctttggaaaagggacacatcttcatgttctgcctactagtggtggcggtggcagcggcggtggtggttcccctggtggcggcggttctggcggtggcggttcctcgagcgaggctgcagtcacccaaagtccaagaagcaaggtggcagtaacaggaggaaaggtgacattgagctgtcaccagactaataaccatgactatatgtactggtatcggcaggacacggggcatgggctgaggctgatccattactcatatgtcgctgacagcacggagaaaggagatatccctgatgggtacaaggcctccagaccaagccaagagaatttctctctcattctggagttggcttccctttctcagacagctgtatatttctgtgccagcagcccccactcctatgaacagtacttcggtcccggcaccaggctcacggttttagaggacctgaacaaggtgttcccacccgaggtcgctgtgtttgagccatcagaagcagagatctcccacacccaaaaggccacactggtgtgcctggccacaggcttcttccctgaccacgtggagctgagctggtgggttaacgggaaggaggtgcacagtggggtcagcacggacccgcagcccctcaaggagcagcccgccctcaatgactccagatactgcctgagcagccgcctgagggtctcggccaccttctggcagaacccccgcaaccacttccgctgtcaagtccagttctacgggctctcggagaatgacgagtggacccaggatagggccaaacctgtcacccagatcgtcagcgccgaggcctggggtagagcagacaactgggtgaatgtaataagtgatttgaaaaaaattgaagatcttattcaatctatgcatattgatgctactttatatacggaaagtgatgttcaccccagttgcaaagtaacagcaatgaagtgctttctcttggagttacaagttatttcacttgagtccggagatgcaagtattcatgatacagtagaaaatctgatcatcctagcaaacgacagtttgtcttctaatgggaatgtaacagaatctggatgcaaagaatgtgaggaactggaggaaaaaaatattaaagaatttttgcagagttttgtacatattgtccaaatgttcatcaacacttcttaa

SEQ ID NO: 39 - protein, 512 aa, Artificial Sequence
  source: /note="Description of Artificial Sequence: Synthetic polypeptide"
MDRLTSSFLLLIVPAYVLAQKVTQTQTSISVMEKTTVTMDCVYETRDSSYFLFWYKQTASGEIVFLIRQDSYKKENATEGHYSLNFQKPKSSIGLIITATQIEDSAVYFCAMRDTNAYKVIFGKGTHLHVLPTSGGGGSGGGGSPGGGGSGGGGSSSEAAVTQSPRSKVAVTGGKVTLSCHQTNNHDYMYWYRQDTGHGLRLIHYSYVADSTEKGDIPDGYKASRPSQENFSLILELASLSQTAVYFCASSPHSYEQYFGPGTRLTVLEDLNKVFPPEVAVFEPSEAEISHTQKATLVCLATGFFPDHVELSWWVNGKEVHSGVSTDPQPLKEQPALNDSRYCLSSRLRVSATFWQNPRNHFRCQVQFYGLSENDEWTQDRAKPVTQIVSAEAWGRADNWVNVISDLKKIEDLIQSMHIDATLYTESDVHPSCKVTAMKCFLLELQVISLESGDASIHDTVENLIILANDSLSSNGNVTESGCKECEELEEKNIKEFLQSFVHIVQMFINTS

SEQ ID NO: 40 - protein, 232 aa, Homo sapiens
EPKSCDKTHTCPPCPAPELLGGPSVFLFPPKPKDTLMISRTPEVTCVVVDVSHEDPEVKFNWYVDGVEVHNAKTKPREEQYNSTYRVVSVLTVLHQDWLNGKEYKCKVSNKALPAPIEKTISKAKGQPREPQVYTLPPSRDELTKNQVSLTCLVKGFYPSDIAVEWESNGQPENNYKTTPPVLDSDGSFFLYSKLTVDKSRWQQGNVFSCSVMHEALHNHYTQKSLSLSPGK

SEQ ID NO: 41 - DNA, 2097 bp, Artificial Sequence
  source: /note="Description of Artificial Sequence: Synthetic polynucleotide"
atggagacagacacactcctgttatgggtactgctgctctgggttccaggttccaccggtcagtcagtgacgcagcccgatgctcgcgtcactgtctctgaaggagcctctctgcagctgagatgcaagtattcctactctgggacaccttatctgttctggtatgtccagtacccgcggcaggggctgcagctgctcctcaagtactattcaggagacccagtggttcaaggagtgaatggcttcgaggctgagttcagcaagagtaactcttccttccacctgcggaaagcctctgtgcactggagcgactctgctgtgtacttctgtgttttgagcgaggatagcaactatcagttgatctggggctctgggaccaagctaattataaagccagacactagtggtggcggtggcagcggcggtggtggttccggtggcggcggttctggcggtggcggttcctcgagcaattcaaaagtcattcagactccaagatatctggtgaaagggcaaggacaaaaagcaaagatgaggtgtatccctgaaaagggacatccagttgtattctggtatcaacaaaataagaacaatgagtttaaatttttgattaactttcagaatcaagaagttcttcagcaaatagacatgactgaaaaacgattctctgctgagtgtccttcaaactcaccttgcagcctagaaattcagtcctctgaggcaggagactcagcactgtacctctgtgccagcagtctgtcagggggcggcacagaagtcttctttggtaaaggaaccaggctcacagttgtagaggacctgaacaaggtgttcccacccgaggtcgctgtgtttgagccatcagaagcagagatctcccacacccaaaaggccacactggtgtgcctggccacaggcttcttccctgaccacgtggagctgagctggtgggttaacgggaaggaggtgcacagtggggtcagcacggacccgcagcccctcaaggagcagcccgccctcaatgactccagatactgcctgagcagccgcctgagggtctcggccaccttctggcagaacccccgcaaccacttccgctgtcaagtccagttctacgggctctcggagaatgacgagtggacccaggatagggccaaacccgtcacccagatcgtcagcgccgaggcctggggtagagcagacatcacgtgccctccccccatgtccgtggaacacgcagacatctgggtcaagagctacagcttgtactccagggagcggtacatttgtaactctggtttcaagcgtaaagccggcacgtccagcctgacggagtgcgtgttgaacaaggccacgaatgtcgcccactggacaacccccagtctcaaatgcattagagagccgaaatcttgtgacaaaactcacacatgcccaccgtgcccagcacctgaactcctggggggaccgtcagtcttcctcttccccccaaaacccaaggacaccctcatgatctcccggacccctgaggtcacatgcgtggtggtggacgtgagccacgaagaccctgaggtcaagttcaactggtacgtggacggcgtggaggtgcataatgccaagacaaagccgcgggaggagcagtacaacagcacgtaccgtgtggtcagcgtcctcaccgtcctgcaccaggactggctgaatggcaaggagtacaagtgcaaggtctccaacaaagccctcccagcccccatcgagaaaaccatctccaaagccaaagggcagccccgagaaccacaggtgtacaccctgcccccatcccgggatgagctgaccaagaaccaggtcagcctgacctgcctggtcaaaggcttctatcccagcgacatcgccgtggagtgggagagcaatgggcagccggagaacaactacaagaccacgcctcccgtgctggactccgacggctccttcttcctctacagcaagctcaccgtggacaagagcaggtggcagcaggggaacgtcttctcatgctccgtgatgcatgaggctctgcacaaccactacacgcagaagagcctctccctgtctcctggtaaataa

SEQ ID NO: 42 - protein, 678 aa, Artificial Sequence [sequence omitted]

SEQ ID NO: 43 - DNA, 1140 bp, Artificial Sequence
  source: /note="Description of Artificial Sequence: Synthetic polynucleotide"
atggattttcaggtgcagattatcagcttcctgctaatcagtgcttcagtcataatgtccagaggacaaattgttctctcccagtctccagcaatcctgtctgcatctccaggggagaaggtcacaatgacttgcagggccagctcaagtgtaagttacatccactggttccagcagaagccaggatcctcccccaaaccctggatttatgccacatccaacctggcttctggagtccctgttcgcttcagtggcagtgggtctgggacttcttactctctcacaatcagcagagtggaggctgaagatgctgccacttattactgccagcagtggactagtaacccacccacgttcggaggggggaccaagctggaaatcaaaagtggaggtggcggatcaggaggcggaggttctggcggaggtgggagtcaggtacaactgcagcagcctggggctgagctggtgaagcctggggcctcagtgaagatgtcctgcaaggcttctggctacacatttaccagttacaatatgcactgggtaaaacagacacctggtcggggcctggaatggattggagctatttatcccggaaatggtgatacttcctacaatcagaagttcaaaggcaaggccacattgactgcagacaaatcctccagcacagcctacatgcagctcagcagcctgacatctgaggactctgcggtctattactgtgcaagatcgacttactacggcggtgactggtacttcaatgtctggggcgcagggaccacggtcaccgtctctgcaaactgggtgaatgtaataagtgatttgaaaaaaattgaagatcttattcaatctatgcatattgatgctactttatatacggaaagtgatgttcaccccagttgcaaagtaacagcaatgaagtgctttctcttggagttacaagttatttcacttgagtccggagatgcaagtattcatgatacagtagaaaatctgatcatcctagcaaacgacagtttgtcttctaatgggaatgtaacagaatctggatgcaaagaatgtgaggaactggaggaaaaaaatattaaagaatttttgcagagttttgtacatattgtccaaatgttcatcaacacttcttaa

SEQ ID NO: 44 - protein, 357 aa, Artificial Sequence
  source: /note="Description of Artificial Sequence: Synthetic polypeptide"
QIVLSQSPAILSASPGEKVTMTCRASSSVSYIHWFQQKPGSSPKPWIYATSNLASGVPVRFSGSGSGTSYSLTISRVEAEDAATYYCQQWTSNPPTFGGGTKLEIKSGGGGSGGGGSGGGGSQVQLQQPGAELVKPGASVKMSCKASGYTFTSYNMHWVKQTPGRGLEWIGAIYPGNGDTSYNQKFKGKATLTADKSSSTAYMQLSSLTSEDSAVYYCARSTYYGGDWYFDVWGAGTTVTVSANWVNVISDLKKIEDLIQSMHIDATLYTESDVHPSCKVTAMKCFLLELQVISLESGDASIHDTVENLIILANDSLSSNGNVTESGCKECEELEEKNIKEFLQSFVHIVQMFINTS

SEQ ID NO: 45 - DNA, 1689 bp, Artificial Sequence
  source: /note="Description of Artificial Sequence: Synthetic polynucleotide"
atggattttcaggtgcagattatcagcttcctgctaatcagtgcttcagtcataatgtccagaggacaaattgttctctcccagtctccagcaatcctgtctgcatctccaggggagaaggtcacaatgacttgcagggccagctcaagtgtaagttacatccactggttccagcagaagccaggatcctcccccaaaccctggatttatgccacatccaacctggcttctggagtccctgttcgcttcagtggcagtgggtctgggacttcttactctctcacaatcagcagagtggaggctgaagatgctgccacttattactgccagcagtggactagtaacccacccacgttcggaggggggaccaagctggaaatcaaaagtggaggtggcggatccggaggtggaggttctggtggaggtgggagtcaggtacaactgcagcagcctggggctgagctggtgaagcctggggcctcagtgaagatgtcctgcaaggcttctggctacacatttaccagttacaatatgcactgggtaaaacagacacctggtcggggcctggaatggattggagctatttatcccggaaatggtgatacttcctacaatcagaagttcaaaggcaaggccacattgactgcagacaaatcctccagcacagcctacatgcagctcagcagcctgacatctgaggactctgcggtctattactgtgcaagatcgacttactacggcggtgactggtacttcratgtctggggcgcagggaccacggtcacmgtctctgcaatcacgtgccctccccccatgtccgtggaacacgcagacatctgggtcaagagctacagcttgtactccagggagcggtacatttgtaactctggtttcaagcgtaaagccggcacgtccagcctgacggagtgcgtgttgaacaaggccacgaatgtcgcccactggacaacccccagtctcaaatgcattagagagccgaaatcttgtgacaaaactcacacatgcccaccgtgcccagcacctgaactcctggggggaccgtcagtcttcctcttccccccaaaacccaaggacaccctcatgatctcccggacccctgaggtcacatgcgtggtggtggacgtgagccacgaagaccctgaggtcaagttcaactggtacgtggacggcgtggaggtgcataatgccaagacaaagccgcgggaggagcagtacaacagcacgtaccgtgtggtcagcgtcctcaccgtcctgcaccaggactggctgaatggcaaggagtacaagtgcaaggtctccaacaaagccctcccagcccccatcgagaaaaccatctccaaagccaaagggcagccccgagaaccacaggtgtacaccctgcccccatcccgggatgagctgaccaagaaccaggtcagcctgacctgcctggtcaaaggcttctatcccagcgacatcgccgtggagtgggagagcaatgggcagccggagaacaactacaagaccacgcctcccgtgctggactccgacggctccttcttcctctacagcaagctcaccgtggacaagagcaggtggcagcaggggaacgtcttctcatgctccgtgatgcatgaggctctgcacaaccactacacgcagaagagcctctccctgtctcctggtaaataa

SEQ ID NO: 46 - protein, 540 aa, Artificial Sequence
  source: /note="Description of Artificial Sequence: Synthetic polypeptide"
QIVLSQSPAILSASPGEKVTMTCRASSSVSYIHWFQQKPGSSPKPWIYATSNLASGVPVRFSGSGSGTSYSLTISRVEAEDAATYYCQQWTSNPPTFGGGTKLEIKSGGGGSGGGGSGGGGSQVQLQQPGAELVKPGASVKMSCKASGYTFTSYNMHWVKQTPGRGLEWIGAIYPGNGDTSYNQKFKGKATLTADKSSSTAYMQLSSLTSEDSAVYYCARSTYYGGDWYFNVWGAGTTVTVSAITCPPPMSVEHADIWVKSYSLYSRERYICNSGFKRKAGTSSLTECVLNKATNVAHWTTPSLKCIREPKSCDKTHTCPPCPAPELLGGPSVFLFPPKPKDTLMISRTPEVTCVVVDVSHEDPEVKFNWYVDGVEVHNAKTKPREEQYNSTYRVVSVLTVLHQDWLNGKEYKCKVSNKALPAPIEKTISKAKGQPREPQVYTLPPSRDELTKNQVSLTCLVKGFYPSDIAVEWESNGQPENNYKTTPPVLDSDGSFFLYSKLTVDKSRWQQGNVFSCSVMHEALHNHYTQKSLSLSPGK

SEQ ID NO: 47 - DNA, 1050 bp, Artificial Sequence
  source: /note="Description of Artificial Sequence: Synthetic polynucleotide"
atggattttcaggtgcagattatcagcttcctgctaatcagtgcttcagtcataatgtccagaggacaaattgttctctcccagtctccagcaatcctgtctgcatctccaggggagaaggtcacaatgacttgcagggccagctcaagtgtaagttacatccactggttccagcagaagccaggatcctcccccaaaccctggatttatgccacatccaacctggcttctggagtccctgttcgcttcagtggcagtgggtctgggacttcttactctctcacaatcagcagagtggaggctgaagatgctgccacttattactgccagcagtggactagtaacccacccacgttcggaggggggaccaagctggaaatcaaacgtacggttgctgcaccatctgtcttcatcttcccgccatctgatgagcagttgaaatctggaactgcctctgttgtgtgcctgctgaataacttctatcccagagaggccaaagtacagtggaaggtggataacgccctccaatcgggtaactcccaggagagtgtcacagagcaggacagcaaggacagcacctacagcctcagcagcaccctgacgctgagcaaagcagactacgagaaacacaaagtctacgcctgcgaagtcacccatcagggcctgagctcgcccgtcacaaagagcttcaacaggggagagtgtaactgggtgaatgtaataagtgatttgaaaaaaattgaagatcttattcaatctatgcatattgatgctactttatatacggaaagtgatgttcaccccagttgcaaagtaacagcaatgaagtgctttctcttggagttacaagttatttcacttgagtccggagatgcaagtattcatgatacagtagaaaatctgatcatcctagcaaacgacagtttgtcttctaatgggaatgtaacagaatctggatgcaaagaatgtgaggaactggaggaaaaaaatattaaagaatttttgcagagttttgtacatattgtccaaatgttcatcaacacttcttaa

SEQ ID NO: 48 - protein, 327 aa, Artificial Sequence
  source: /note="Description of Artificial Sequence: Synthetic polypeptide"
QIVLSQSPAILSASPGEKVTMTCRASSSVSYIHWFQQKPGSSPKPWIYATSNLASGVPVRFSGSGSGTSYSLTISRVEAEDAATYYCQQWTSNPPTFGGGTKLEIKRTVAAPSVFIFPPSDEQLKSGTASVVCLLNNFYPREAKVQWKVDNALQSGNSQESVTEQDSKDSTYSLSSTLTLSKADYEKHKVYACEVTHQGLSSPVTKSFNRGECNWVNVISDLKKIEDLIQSMHIDATLYTESDVHPSCKVTAMKCFLLELQVISLESGDASIHDTVENLIILANDSLSSNGNVTESGCKECEELEEKNIKEFLQSFVHIVQMFINTS

SEQ ID NO: 49 - DNA, 1608 bp, Artificial Sequence
  source: /note="Description of Artificial Sequence: Synthetic polynucleotide"
atgggttggagtctcatcttgctcttccttgtcgctgttgctacacgtgtcctgtcccaggtacaactgcagcagcctggggctgagctggtgaagcctggggcctcagtgaagatgtcctgcaaggcttctggctacacatttaccagttacaatatgcactgggtaaaacagacacctggtcggggcctggaatggattggagctatttatcccggaaatggtgatacttcctacaatcagaagttcaaaggcaaggccacattgactgcagacaaatcctccagcacagcctacatgcagctcagcagcctgacatctgaggactctgcggtctattactgtgcaagatcgacttactacggcggtgactggtacttcgatgtctggggcgcagggaccacggtcaccgtctctgcagctagcaccaagggcccatcggtcttccccctggcaccctcctccaagagcacctctgggggcacagcggccctgggctgcctggtcaaggactacttccccgaaccggtgacggtgtcgtggaactcaggcgccctgaccagcggcgtgcacaccttcccggctgtcctacagtcctcaggactctactccctcagcagcgtggtgaccgtgccctccagcagcttgggcacccagacctacatctgcaacgtgaatcacaagcccagcaacaccaaggtggacaagaaagttatcacgtgccctccccccatgtccgtggaacacgcagacatctgggtcaagagctacagcttgtactccagggagcggtacatttgtaactctggtttcaagcgtaaagccggcacgtccagcctgacggagtgcgtgttgaacaaggccacgaatgtcgcccactggacaacccccagtctcaaatgcattagagagcccaaatcttgtgacaaaactcacacatgcccaccgtgcccagcacctgaactcctggggggaccgtcagtcttcctcttccccccaaaacccaaggacaccctcatgatctcccggacccctgaggtcacatgcgtggtggtggacgtgagccacgaagaccctgaggtcaagttcaactggtacgtggacggcgtggaggtgcataatgccaagacaaagccgcgggaggagcagtacaacagcacgtaccgtgtggtcagcgtcctcaccgtcctgcaccaggactggctgaatggcaaggagtacaagtgcaaggtctccaacaaagccctcccagcccccatcgagaaaaccatctccaaagccaaagggcagccccgagaaccacaggtgtacaccctgcccccatcccgggatgagctgaccaagaaccaggtcagcctgacctgcctggtcaaaggcttctatcccagcgacatcgccgtggagtgggagagcaatgggcagccggagaacaactacaagaccacgcctcccgtgctggactccgacggctccttcttcctctacagcaagctcaccgtggacaagagcaggtggcagcaggggaacgtcttctcatgctccgtgatgcatgaggctctgcacaaccactacacgcagaagagcctctccctgtctcctggtaaataa

SEQ ID NO: 50 - protein, 516 aa, Artificial Sequence
  source: /note="Description of Artificial Sequence: Synthetic polypeptide"
QVQLQQPGAELVKPGASVKMSCKASGYTFTSYNMHWVKQTPGRGLEWIGAIYPGNGDTSYNQKFKGKATLTADKSSSTAYMQLSSLTSEDSAVYYCARSTYYGGDWYFDVWGAGTTVTVSAASTKGPSVFPLAPSSKSTSGGTAALGCLVKDYFPEPVTVSWNSGALTSGVHTFPAVLQSSGLYSLSSVVTVPSSSLGTQTYICNVNHKPSNTKVDKKVITCPPPMSVEHADIWVKSYSLYSRERYICNSGFKRKAGTSSLTECVLNKATNVAHWTTPSLKCIREPKSCDKTHTCPPCPAPELLGGPSVFLFPPKPKDTLMISRTPEVTCVVVDVSHEDPEVKFNWYVDGVEVHNAKTKPREEQYNSTYRVVSVLTVLHQDWLNGKEYKCKVSNKALPAPIEKTISKAKGQPREPQVYTLPPSRDELTKNQVSLTCLVKGFYPSDIAVEWESNGQPENNYKTTPPVLDSDGSFFLYSKLTVDKSRWQQGNVFSCSVMHEALHNHYTQKSLSLSPGK

SEQ ID NO: 51 - protein, 114 aa, Homo sapiens
NWVNVISDLKKIEDLIQSMHIDATLYTESDVHPSCKVTAMKCFLLELQVISLESGDASIHDTVENLIILANNSLSSNGNVTESGCKECEELEEKNIKEFLQSFVHIVQMFINTS